European Patent Specification EP 3 645 557 B1, published October 23, 2024. Title: TREATMENT OF NERVOUS SYSTEM INJURY AND NEURODEGENERATIVE DISORDERS AND RELATED CONDITIONS. Applicant: THE CLEVELAND CLINIC FOUNDATION. The sequence listing filed with the application follows.

SEQUENCE LISTING (90 sequences)

SEQ ID NO: 1 - protein, 11 aa, Artificial Sequence
  Synthetic
YGRKKRRQRRR

SEQ ID NO: 2 - protein, 19 aa, Artificial Sequence
  Synthetic
PKPRVTWNKKGKKVNSQRF

SEQ ID NO: 3 - protein, 14 aa, Artificial Sequence
  Synthetic
KFERQKILDQRFFE

SEQ ID NO: 4 - protein, 46 aa, Artificial Sequence
  Synthetic
NYGRKKRRQRRRPKPRVTWNKKGKKVNSQRFKFERQKILDQRFFEC

SEQ ID NO: 5 - protein, 12 aa, Artificial Sequence
  Synthetic
YGRKKRRQRRRC

SEQ ID NO: 6 - protein, 13 aa, Artificial Sequence
  Synthetic
YGRKKRRQRRRGC

SEQ ID NO: 7 - protein, 13 aa, Artificial Sequence
  Synthetic
CAYGRKKRRQRRR

SEQ ID NO: 8 - protein, 33 aa, Artificial Sequence
  Synthetic
YGRKKRRQRRRYGRKKRRQRRRYGRKKRRQRRR

SEQ ID NO: 9 - protein, 10 aa, Artificial Sequence
  Synthetic
GRKKRRQRRR

SEQ ID NO: 10 - protein, 11 aa, Artificial Sequence
  Synthetic
GRKKRRQRRRG

SEQ ID NO: 11 - protein, 12 aa, Artificial Sequence
  Synthetic
GRKKRRQRRRCG

SEQ ID NO: 12 - protein, 12 aa, Artificial Sequence
  Synthetic
GRKKRRQRRRPP

SEQ ID NO: 13 - protein, 13 aa, Artificial Sequence
  Synthetic
GRKKRRQRRRPPQ

SEQ ID NO: 14 - protein, 14 aa, Artificial Sequence
  Synthetic
GRKKRRQRRRPPQC

SEQ ID NO: 15 - protein, 9 aa, Artificial Sequence
  Synthetic
RKKRRQRRR

SEQ ID NO: 16 - protein, 9 aa, Artificial Sequence
  Synthetic
RKKRRQRRR

SEQ ID NO: 17 - protein, 9 aa, Artificial Sequence
  Synthetic
RRRQRRKKR

SEQ ID NO: 18 - protein, 9 aa, Artificial Sequence
  Synthetic
RRRQRRKKR

SEQ ID NO: 19 - protein, 13 aa, Artificial Sequence
  Synthetic
GRRRRRRRRRPPQ

SEQ ID NO: 20 - protein, 19 aa, Artificial Sequence
  Synthetic
TRQARRNRRRRWRERQRGC

SEQ ID NO: 21 - protein, 15 aa, Artificial Sequence
  Synthetic
TRRQRTRRARRNRGC

SEQ ID NO: 22 - protein, 21 aa, Artificial Sequence
  Synthetic
KLTRAQRRAAARKNKRNTRGC

SEQ ID NO: 23 - protein, 15 aa, Artificial Sequence
  Synthetic
RRRRNRTRRNRRRVR

SEQ ID NO: 24 - protein, 8 aa, Artificial Sequence
  Synthetic
RRRRRRGC

SEQ ID NO: 25 - protein, 10 aa, Artificial Sequence
  Synthetic
RRRRRRRRGC

SEQ ID NO: 26 - protein, 21 aa, Artificial Sequence
  Synthetic
KETWWETWWTEWSQPKKKRKV

SEQ ID NO: 27 - protein, 16 aa, Artificial Sequence
  Synthetic
RQILIWFQNRRMKWKK

SEQ ID NO: 28 - protein, 5 aa, Artificial Sequence
  Synthetic
KFERQ

SEQ ID NO: 29 - protein, 5 aa, Artificial Sequence
  Synthetic
KFERQ

SEQ ID NO: 30 - protein, 5 aa, Artificial Sequence
  Synthetic
QKILD

SEQ ID NO: 31 - protein, 5 aa, Artificial Sequence
  Synthetic
QRFFE

SEQ ID NO: 32 - protein, 9 aa, Artificial Sequence
  Synthetic
KFERQKILD

SEQ ID NO: 33 - protein, 10 aa, Artificial Sequence
  Synthetic
QKILDQRFFE

SEQ ID NO: 34 - protein, 9 aa, Artificial Sequence
  Synthetic
KFERQRFFE

SEQ ID NO: 35 - protein, 7 aa, Artificial Sequence
  Synthetic
QRFFERQ

SEQ ID NO: 36 - protein, 7 aa, Artificial Sequence
  Synthetic
QRKFERQ

SEQ ID NO: 37 - protein, 5 aa, Artificial Sequence
  Synthetic
KKGKK

SEQ ID NO: 38 - protein, 7 aa, Artificial Sequence
  Synthetic
NKKGKKV

SEQ ID NO: 39 - protein, 9 aa, Artificial Sequence
  Synthetic
NKKGKKVNS

SEQ ID NO: 40 - protein, 11 aa, Artificial Sequence
  Synthetic
KKGKKVNSQRF

SEQ ID NO: 41 - protein, 15 aa, Artificial Sequence
  Synthetic
RVTWNKKGKKVNSQR

SEQ ID NO: 42 - protein, 20 aa, Artificial Sequence
  Synthetic
PKPRVTWNKKGKKVNSQRFE

SEQ ID NO: 43 - protein, 22 aa, Artificial Sequence
  Synthetic
TGDPKPRVTWNKKGKKVNSQRF

SEQ ID NO: 44 - protein, 23 aa, Artificial Sequence
  Synthetic
TGDPKPRVTWNKKGKKVNSQRFE

SEQ ID NO: 45 - protein, 19 aa, Artificial Sequence
  Synthetic
PKPRVTWNRKGKKVNSQRF

SEQ ID NO: 46 - protein, 19 aa, Artificial Sequence
  Synthetic
PKPRVTWNRRGKKVNSQRF

SEQ ID NO: 47 - protein, 19 aa, Artificial Sequence
  Synthetic
PKPRVTWNRRGRKVNSQRF

SEQ ID NO: 48 - protein, 19 aa, Artificial Sequence
  Synthetic
PKPRVTWNRRGRRVNSQRF

SEQ ID NO: 49 - protein, 19 aa, Artificial Sequence
  Synthetic
PKPRVTWNKRGKKVNSQRF

SEQ ID NO: 50 - protein, 19 aa, Artificial Sequence
  Synthetic
PKPRVTWNKRGRKVNSQRF

SEQ ID NO: 51 - protein, 19 aa, Artificial Sequence
  Synthetic
PKPRVTWNKRGRRVNSQRF

SEQ ID NO: 52 - protein, 19 aa, Artificial Sequence
  Synthetic
PKPRVTWNKKGRKVNSQRF

SEQ ID NO: 53 - protein, 19 aa, Artificial Sequence
  Synthetic
PKPRVTWNKKGRRVNSQRF

SEQ ID NO: 54 - protein, 10 aa, Artificial Sequence
  Synthetic
  misc_feature (3)..(4): pY is phosphorylated tyrosine
VQPYSTVVHS

SEQ ID NO: 55 - protein, 9 aa, Artificial Sequence
  Synthetic
VQYSTVVHS

SEQ ID NO: 56 - protein, 10 aa, Artificial Sequence
  Synthetic
  misc_feature (3)..(4): pY is phosphorylated tyrosine
VEPYSTVVHS

SEQ ID NO: 57 - protein, 9 aa, Artificial Sequence
  Synthetic
VEYSTVVHS

SEQ ID NO: 58 - protein, 9 aa, Artificial Sequence
  Synthetic
  misc_feature (2)..(2): x is any amino acid
  misc_feature (3)..(4): pY is phosphorylated tyrosine
  misc_feature (5)..(6): x is any amino acid
  misc_feature (9)..(9): x is any amino acid
VXPYXXVVX

SEQ ID NO: 59 - protein, 9 aa, Artificial Sequence
  Synthetic
  misc_feature (2)..(2): x is any amino acid
  misc_feature (3)..(4): pY is phosphorylated tyrosine
  misc_feature (5)..(6): x is any amino acid
  misc_feature (9)..(9): x is any amino acid
VXPYXXLVX

SEQ ID NO: 60 - protein, 9 aa, Artificial Sequence
  Synthetic
  misc_feature (2)..(2): x is any amino acid
  misc_feature (3)..(4): pY is phosphorylated tyrosine
  misc_feature (5)..(6): x is any amino acid
  misc_feature (9)..(9): x is any amino acid
VXPYXXVLX

SEQ ID NO: 61 - protein, 9 aa, Artificial Sequence
  Synthetic
  misc_feature (2)..(2): x is any amino acid
  misc_feature (3)..(4): pY is phosphorylated tyrosine
  misc_feature (5)..(6): x is any amino acid
  misc_feature (9)..(9): x is any amino acid
LXPYXXVVX

SEQ ID NO: 62 - protein, 9 aa, Artificial Sequence
  Synthetic
  misc_feature (2)..(2): x is any amino acid
  misc_feature (3)..(4): pY is phosphorylated tyrosine
  misc_feature (5)..(6): x is any amino acid
  misc_feature (9)..(9): x is any amino acid
VXPYXXLLX

SEQ ID NO: 63 - protein, 9 aa, Artificial Sequence
  Synthetic
  misc_feature (2)..(2): x is any amino acid
  misc_feature (3)..(4): pY is phosphorylated tyrosine
  misc_feature (5)..(6): x is any amino acid
  misc_feature (9)..(9): x is any amino acid
LXPYXXVLX

SEQ ID NO: 64 - protein, 9 aa, Artificial Sequence
  Synthetic
  misc_feature (2)..(2): x is any amino acid
  misc_feature (3)..(4): pY is phosphorylated tyrosine
  misc_feature (5)..(6): x is any amino acid
  misc_feature (9)..(9): x is any amino acid
LXPYXXLVX

SEQ ID NO: 65 - protein, 9 aa, Artificial Sequence
  Synthetic
  misc_feature (2)..(2): x is any amino acid
  misc_feature (3)..(4): pY is phosphorylated tyrosine
  misc_feature (5)..(6): x is any amino acid
  misc_feature (9)..(9): x is any amino acid
LXPYXXLLX

SEQ ID NO: 66 - protein, 8 aa, Artificial Sequence
  Synthetic
  misc_feature (2)..(2): x is any amino acid
  misc_feature (4)..(5): x is any amino acid
  misc_feature (8)..(8): x is any amino acid
VXYXXVVX

SEQ ID NO: 67 - protein, 8 aa, Artificial Sequence
  Synthetic
  misc_feature (2)..(2): x is any amino acid
  misc_feature (4)..(5): x is any amino acid
  misc_feature (8)..(8): x is any amino acid
VXYXXLVX

SEQ ID NO: 68 - protein, 8 aa, Artificial Sequence
  Synthetic
  misc_feature (2)..(2): x is any amino acid
  misc_feature (4)..(5): x is any amino acid
  misc_feature (8)..(8): x is any amino acid
VXYXXVLX

SEQ ID NO: 69 - protein, 8 aa, Artificial Sequence
  Synthetic
  misc_feature (2)..(2): x is any amino acid
  misc_feature (4)..(5): x is any amino acid
  misc_feature (8)..(8): x is any amino acid
LXYXXVVX

SEQ ID NO: 70 - protein, 8 aa, Artificial Sequence
  Synthetic
  misc_feature (2)..(2): x is any amino acid
  misc_feature (4)..(5): x is any amino acid
  misc_feature (8)..(8): x is any amino acid
VXYXXLLX

SEQ ID NO: 71 - protein, 8 aa, Artificial Sequence
  Synthetic
  misc_feature (2)..(2): x is any amino acid
  misc_feature (4)..(5): x is any amino acid
  misc_feature (8)..(8): x is any amino acid
LXYXXVLX

SEQ ID NO: 72 - protein, 8 aa, Artificial Sequence
  Synthetic
  misc_feature (2)..(2): x is any amino acid
  misc_feature (4)..(5): x is any amino acid
  misc_feature (8)..(8): x is any amino acid
LXYXXLVX

SEQ ID NO: 73 - protein, 8 aa, Artificial Sequence
  Synthetic
  misc_feature (2)..(2): x is any amino acid
  misc_feature (4)..(5): x is any amino acid
  misc_feature (8)..(8): x is any amino acid
LXYXXLLX

SEQ ID NO: 74 - protein, 10 aa, Artificial Sequence
  Synthetic
  misc_feature (2)..(2): x is any amino acid
  misc_feature (3)..(4): pY is phosphorylated tyrosine
  misc_feature (5)..(6): x is any amino acid
  misc_feature (9)..(9): x is any amino acid
VXPYXXVVXS

SEQ ID NO: 75 - protein, 10 aa, Artificial Sequence
  Synthetic
  misc_feature (2)..(2): x is any amino acid
  misc_feature (3)..(4): pY is phosphorylated tyrosine
  misc_feature (5)..(6): x is any amino acid
  misc_feature (9)..(9): x is any amino acid
VXPYXXLVXS

SEQ ID NO: 76 - protein, 10 aa, Artificial Sequence
  Synthetic
  misc_feature (2)..(2): x is any amino acid
  misc_feature (3)..(4): pY is phosphorylated tyrosine
  misc_feature (5)..(6): x is any amino acid
  misc_feature (9)..(9): x is any amino acid
VXPYXXVLXS

SEQ ID NO: 77 - protein, 10 aa, Artificial Sequence
  Synthetic
  misc_feature (2)..(2): x is any amino acid
  misc_feature (3)..(4): pY is phosphorylated tyrosine
  misc_feature (5)..(6): x is any amino acid
  misc_feature (9)..(9): x is any amino acid
LXPYXXVVXS

SEQ ID NO: 78 - protein, 10 aa, Artificial Sequence
  Synthetic
  misc_feature (2)..(2): x is any amino acid
  misc_feature (3)..(4): pY is phosphorylated tyrosine
  misc_feature (5)..(6): x is any amino acid
  misc_feature (9)..(9): x is any amino acid
VXPYXXLLXS

SEQ ID NO: 79 - protein, 10 aa, Artificial Sequence
  Synthetic
  misc_feature (2)..(2): x is any amino acid
  misc_feature (3)..(4): pY is phosphorylated tyrosine
  misc_feature (5)..(6): x is any amino acid
  misc_feature (9)..(9): x is any amino acid
LXPYXXVLXS

SEQ ID NO: 80 - protein, 10 aa, Artificial Sequence
  Synthetic
  misc_feature (2)..(2): x is any amino acid
  misc_feature (3)..(4): pY is phosphorylated tyrosine
  misc_feature (5)..(6): x is any amino acid
  misc_feature (9)..(9): x is any amino acid
LXPYXXLVXS

SEQ ID NO: 81 - protein, 10 aa, Artificial Sequence
  Synthetic
  misc_feature (2)..(2): x is any amino acid
  misc_feature (3)..(4): pY is phosphorylated tyrosine
  misc_feature (5)..(6): x is any amino acid
  misc_feature (9)..(9): x is any amino acid
LXPYXXLLXS

SEQ ID NO: 82 - protein, 16 aa, Artificial Sequence
  Synthetic
STASTVEPYSTVVHSG

SEQ ID NO: 83 - protein, 15 aa, Artificial Sequence
  Synthetic
STASTVEPYSTVVHS

SEQ ID NO: 84 - protein, 14 aa, Artificial Sequence
  Synthetic
STASTVQPYSTVVH

SEQ ID NO: 85 - protein, 13 aa, Artificial Sequence
  Synthetic
STASTVQPYSTVV

SEQ ID NO: 86 - protein, 16 aa, Artificial Sequence
  Synthetic
STASTVQPYSTVVHSG

SEQ ID NO: 87 - protein, 15 aa, Artificial Sequence
  Synthetic
STASTVQPYSTVVHS

SEQ ID NO: 88 - protein, 14 aa, Artificial Sequence
  Synthetic
STASTVQPYSTVVH

SEQ ID NO: 89 - protein, 13 aa, Artificial Sequence
  Synthetic
STASTVQPYSTVV

SEQ ID NO: 90 - protein, 35 aa, Artificial Sequence
  Synthetic
YGRKKRRQRRRVQPYSTVVHSKFERQKILDQRFFE